European Patent Specification EP 3 175 023 B1, published February 19, 2025. Title: SYSTEMS AND METHODS FOR DETERMINING NUCLEIC ACIDS. Applicant: President and Fellows of Harvard College. Application Not Yet Assigned. The sequence listing filed with the application follows.

SEQUENCE LISTING (40 sequences)

SEQ ID NO: 1 - DNA, 120 bp, Artificial Sequence
  Synthetic Polynucleotide
gttggcgacgaaagcactgcgattggaaccgtcccaagcgttgcgcttaatggatcatcaattttgtctcactacgacggtcaatcgcgctgcatacttgcgtcggtcggacaaacgagg

SEQ ID NO: 2 - DNA, 30 bp, Artificial Sequence
  Synthetic Polynucleotide
cgcaacgcttgggacggttccaatcggatc

SEQ ID NO: 3 - DNA, 30 bp, Artificial Sequence
  Synthetic Polynucleotide
cgaatgctctggcctcgaacgaacgatagc

SEQ ID NO: 4 - DNA, 30 bp, Artificial Sequence
  Synthetic Polynucleotide
acaaatccgaccagatcggacgatcatggg

SEQ ID NO: 5 - DNA, 30 bp, Artificial Sequence
  Synthetic Polynucleotide
caagtatgcagcgcgattgaccgtctcgtt

SEQ ID NO: 6 - DNA, 30 bp, Artificial Sequence
  Synthetic Polynucleotide
tgcgtcgtctggctagcacggcacgcaaat

SEQ ID NO: 7 - DNA, 30 bp, Artificial Sequence
  Synthetic Polynucleotide
aagtcgtacgccgatgcgcagcaattcact

SEQ ID NO: 8 - DNA, 30 bp, Artificial Sequence
  Synthetic Polynucleotide
cgaaacatcggccacggtcccgttgaactt

SEQ ID NO: 9 - DNA, 30 bp, Artificial Sequence
  Synthetic Polynucleotide
acgaatccaccgtccagcgcgtcaaacaga

SEQ ID NO: 10 - DNA, 30 bp, Artificial Sequence
  Synthetic Polynucleotide
cgcgaaatccccgtaacgagcgtcccttgc

SEQ ID NO: 11 - DNA, 30 bp, Artificial Sequence
  Synthetic Polynucleotide
gcatgagttgcctggcgttgcgacgactaa

SEQ ID NO: 12 - DNA, 30 bp, Artificial Sequence
  Synthetic Polynucleotide
ccgtcgtctccggtccaccgttgcgcttac

SEQ ID NO: 13 - DNA, 30 bp, Artificial Sequence
  Synthetic Polynucleotide
ggccaatggcccaggtccgtcacgcaattt

SEQ ID NO: 14 - DNA, 30 bp, Artificial Sequence
  Synthetic Polynucleotide
ttgatcgaatcggagcgtagcggaatctgc

SEQ ID NO: 15 - DNA, 30 bp, Artificial Sequence
  Synthetic Polynucleotide
cgcgcggatccgcttgtcgggaacggatac

SEQ ID NO: 16 - DNA, 30 bp, Artificial Sequence
  Synthetic Polynucleotide
gcctcgattacgacggatgtaattcggccg

SEQ ID NO: 17 - DNA, 30 bp, Artificial Sequence
  Synthetic Polynucleotide
gcccgtattcccgcttgcgagtagggcaat

SEQ ID NO: 18 - DNA, 20 bp, Artificial Sequence
  Synthetic Polynucleotide
gttggtcggcacttgggtgc

SEQ ID NO: 19 - DNA, 20 bp, Artificial Sequence
  Synthetic Polynucleotide
cgatgcgccaattccggttc

SEQ ID NO: 20 - DNA, 20 bp, Artificial Sequence
  Synthetic Polynucleotide
cgcgggctatatgcgaaccg

SEQ ID NO: 21 - DNA, 40 bp, Artificial Sequence
  Synthetic Polynucleotide
taatacgactcactatagggaaagccggttcatccggtgg

SEQ ID NO: 22 - DNA, 40 bp, Artificial Sequence
  Synthetic Polynucleotide
taatacgactcactatagggtgatcatcgctcgcgggttg

SEQ ID NO: 23 - DNA, 39 bp, Artificial Sequence
  Synthetic Polynucleotide
taatacgactcactatagggcgtggagggcatacaacgc

SEQ ID NO: 24 - DNA, 30 bp, Artificial Sequence; identical to SEQ ID NO: 2
  Synthetic Polynucleotide
  misc_feature (30)..(30): Cytosine is modified by 3' Cy5 Sp

SEQ ID NO: 25 - DNA, 30 bp, Artificial Sequence; identical to SEQ ID NO: 3
  Synthetic Polynucleotide
  misc_feature (30)..(30): Cytosine is modified by 3' Cy5 Sp

SEQ ID NO: 26 - DNA, 30 bp, Artificial Sequence; identical to SEQ ID NO: 4
  Synthetic Polynucleotide
  misc_feature (30)..(30): Guanine is modified by 3' Cy5 Sp

SEQ ID NO: 27 - DNA, 30 bp, Artificial Sequence; identical to SEQ ID NO: 5
  Synthetic Polynucleotide
  misc_feature (30)..(30): Thymine is modified by 3' Cy5 Sp

SEQ ID NO: 28 - DNA, 30 bp, Artificial Sequence
  Synthetic Polynucleotide
  misc_feature (30)..(30): Cytosine is modified by 3' Cy5 Sp
gcgggaagcacgtggattagggcatcgacc

SEQ ID NO: 29 - DNA, 30 bp, Artificial Sequence; identical to SEQ ID NO: 7
  misc_feature (30)..(30): Thymine is modified by 3' Cy5 Sp
  Synthetic Polynucleotide

SEQ ID NO: 30 - DNA, 30 bp, Artificial Sequence; identical to SEQ ID NO: 8
  Synthetic Polynucleotide
  misc_feature (30)..(30): Thymine is modified by 3' Cy5 Sp

SEQ ID NO: 31 - DNA, 30 bp, Artificial Sequence; identical to SEQ ID NO: 9
  Synthetic Polynucleotide
  misc_feature (30)..(30): Adenine is modified by 3' Cy5 Sp

SEQ ID NO: 32 - DNA, 30 bp, Artificial Sequence; identical to SEQ ID NO: 10
  Synthetic Polynucleotide
  misc_feature (30)..(30): Cytosine is modified by 3' Cy5 Sp

SEQ ID NO: 33 - DNA, 30 bp, Artificial Sequence; identical to SEQ ID NO: 11
  Synthetic Polynucleotide
  misc_feature (30)..(30): Adenine is modified by 3' Cy5 Sp

SEQ ID NO: 34 - DNA, 30 bp, Artificial Sequence; identical to SEQ ID NO: 12
  Synthetic Polynucleotide
  misc_feature (30)..(30): Cytosine is modified by 3' Cy5 Sp

SEQ ID NO: 35 - DNA, 30 bp, Artificial Sequence; identical to SEQ ID NO: 13
  Synthetic Polynucleotide
  misc_feature (30)..(30): Thymine is modified by 3' Cy5 Sp

SEQ ID NO: 36 - DNA, 30 bp, Artificial Sequence; identical to SEQ ID NO: 14
  Synthetic Polynucleotide
  misc_feature (30)..(30): Cytosine is modified by 3' Cy5 Sp

SEQ ID NO: 37 - DNA, 30 bp, Artificial Sequence; identical to SEQ ID NO: 15
  Synthetic Polynucleotide
  misc_feature (30)..(30): Cytosine is modified by 3' Cy5 Sp

SEQ ID NO: 38 - DNA, 30 bp, Artificial Sequence; identical to SEQ ID NO: 16
  Synthetic Polynucleotide
  misc_feature (30)..(30): Guanine is modified by 3' Cy5 Sp

SEQ ID NO: 39 - DNA, 30 bp, Artificial Sequence; identical to SEQ ID NO: 17
  Synthetic Polynucleotide
  misc_feature (30)..(30): Thymine is modified by 3' Cy5 Sp

SEQ ID NO: 40 - DNA, 20 bp, Artificial Sequence
  Synthetic Polynucleotide
cgggtttagcgccggaaatg